European Patent Application EP 4 755 906 A2, published June 10, 2026. Title: DUAL CSF-1 IL-10 CYTOKINE. Applicant: ORIKINE BIO SL. Application WO. The sequence listing filed with the application follows.

SEQUENCE LISTING (74 sequences)

SEQ ID NO: 1 - protein, 301 aa, synthetic construct
MTQSENSCTHFPGNLPNMLRDLRDAFSRVKTFFQMKDQLDNLLLKESLLEDFKGYLGCQALSEMIQFYLEEVMPQAENQEPDIKAHVNSLGENLKTLRLRLRRCHRFLPCENKSKAVEQVKNAFNKLQEKGIYKAMSEFDIFINYIEAYMTMNNGGLDYLPNMLRDLRDAFSRVKTFFQMKDQLDNLLLKESLLEDFKGYLGCQALSEMIQFYLEEVMPQAENQDPDIKAHVNSLGENLKTLRLRLRRNHRFLPCENKSKAVEQVKNAFNKLQEKGIYKAMSEFDIFINYIEAYMTMKIRN

SEQ ID NO: 2 - protein, 297 aa, synthetic construct
MTQSENSCTHFPGNLPNMLRDLRDAFSRVKTFFQMKDQLDNLLLKESLLEDFKGYLGCQALSEMIQFYLEEVMPQAENQDPDIKAHVNSLGENLKTLRLRLRRCHRFLPCENKSKAVEQVKNAFNKLQEKGIYKAMSEFDIFINYIEAYMTMNFGGLDYLPNMLRDLRDAFSRVKTFFQMKDQLDNLLLKESLLEDFKGYLGCQALSEMIQFYLEEVMPQAENQDPDIKAHVNSLGENLKTLRLRLRRCHRFLPCENKSKAVEQVKNAFNKLQEKGIYKAMSEFDIFINYIEAYMTM

SEQ ID NO: 3 - protein, 295 aa, synthetic construct
MTQSENSCTHFPGNLPNMLRDLRDAFSRVKTFFQMKDQLDNLLLKESLLEDFKGYLGCQALSEMIQFYLEEVMPQAENQDPDIKAHVNSLGENLKTLRLRLRRCHRFLPCENKSKAVEQVKNAFNKLQEKGIYKAMSEFDIFINYIEAYLYKTITPEFANMLRDLRDAFSRVKTFFQMKDQLDNLLLKESLLEDFKGYLGCQALSEMIQFYLEEVMPQAENQDPDIKAHVNSLGENLKTLRLRLRRCHRFLPCENKSKAVEQVKNAFNKLQEKGIYKAMSEFDIFINYIEAYMTM

SEQ ID NO: 4 - protein, 296 aa, synthetic construct
MTQSENSCTHFPGNLPNMLRDLRDAFSRVKTFFQMKDQLDNLLLKESLLEDFKGYLGCQALSEMIQFYLEEVMPQAENQDPDIKAHVNSLGENLKTLRLRLRRCHRFLPCENKSKAVEQVKNAFNKLQEKGIYKAMSEFDIFINYIEAKDKDIRDGDELANMLRDLRDAFSRVKTFFQMKDQLDNLLLKESLLEDFKGYLGCQALSEMIQFYLEEVMPQAENQDPDIKAHVNSLGENLKTLRLRLRRCHRFLPCENKSKAVEQVKNAFNKLQEKGIYKAMSEFDIFINYIEAYMTM

SEQ ID NO: 5 - protein, 290 aa, synthetic construct
NKSKAVEQVKNAFNKLQEKGIYKAMSEFDIFINYIEAYMTMNNGGLDYLPNMLRDLRDAFSRVKTFFQMKDQLDNLLLKESLLEDFKGYLGCQALSEMIQFYLEEVMPQAENQDPDIKAHVNSLGENLKTLRLRLRRNHRFLPCENKSKAVEQVKNAFNKLQEKGIYKAMSEFDIFINYIEAYMTMNNGGLDYLPNMLRDLRDAFSRVKTFFQMKDQLDNLLLKESLLEDFKGYLGCQALSEMIQFYLEEVMPQAENQDPDIKAHVNSLGENLKTLRLRLRRNHRFLPCE

SEQ ID NO: 6 - protein, 290 aa, synthetic construct
EKGIYKAMSEFDIFINYIEAYMTMNNGGLDYLPNMLRDLRDAFSRVKTFFQMKDQLDNLLLKESLLEDFKGYLGCQALSEMIQFYLEEVMPQAENQDPDIKAHVNSLGENLKTLRLRLRRNHRFLPCENKSKAVEQVKNAFNKLQEKGIYKAMSEFDIFINYIEAYMTMNNGGLDYLPNMLRDLRDAFSRVKTFFQMKDQLDNLLLKESLLEDFKGYLGCQALSEMIQFYLEEVMPQAENQDPDIKAHVNSLGENLKTLRLRLRRNHRFLPCENKSKAVEQVKNAFNKLQ

SEQ ID NO: 7 - protein, 290 aa, synthetic construct
GYLGCQALSEMIQFYLEEVMPQAENQDPDIKAHVNSLGENLKTLRLRLRRNHRFLPCENKSKAVEQVKNAFNKLQEKGIYKAMSEFDIFINYIEAYMTMNNGGLDYLPNMLRDLRDAFSRVKTFFQMKDQLDNLLLKESLLEDFKGYLGCQALSEMIQFYLEEVMPQAENQDPDIKAHVNSLGENLKTLRLRLRRNHRFLPCENKSKAVEQVKNAFNKLQEKGIYKAMSEFDIFINYIEAYMTMNNGGLDYLPNMLRDLRDAFSRVKTFFQMKDQLDNLLLKESLLEDFK

SEQ ID NO: 8 - protein, 290 aa, synthetic construct
DIKAHVNSLGENLKTLRLRLRRNHRFLPCENKSKAVEQVKNAFNKLQEKGIYKAMSEFDIFINYIEAYMTMNNGGLDYLPNMLRDLRDAFSRVKTFFQMKDQLDNLLLKESLLEDFKGYLGCQALSEMIQFYLEEVMPQAENQDPDIKAHVNSLGENLKTLRLRLRRNHRFLPCENKSKAVEQVKNAFNKLQEKGIYKAMSEFDIFINYIEAYMTMNNGGLDYLPNMLRDLRDAFSRVKTFFQMKDQLDNLLLKESLLEDFKGYLGCQALSEMIQFYLEEVMPQAENQDP

SEQ ID NO: 9 - protein, 155 aa, synthetic construct
KACVRTFYETPLQLLEKVKNVFNETKNLLDKDWNIFSKNCNNSFNECEDQDRRQPGTKTTGKVSEYCSHMIGSGHLQSLQRLIDSQMETSCQITFEFVDQEQLKDPVCYLKKAFLLVQDIMEDTMRFRDNTPNAIAIVQLQELSLRLKSCFTKDY

SEQ ID NO: 10 - protein, 158 aa, synthetic construct
KACVRTFYETPLQLLEKVKNVFNETKNLLDKDWNIFSKNCNNSFAECGKPPQYIDRHTQPGQPNATSEYCSHMIGSGHLQSLQRLIDSQMETSCQITFEFVDQEQLKDPVCYLKKAFLLVQDIMEDTMRFRDNTPNAIAIVQLQELSLRLKSCFTKDY

SEQ ID NO: 11 - protein, 160 aa, Homo sapiens
SPGQGTQSENSCTHFPGNLPNMLRDLRDAFSRVKTFFQMKDQLDNLLLKESLLEDFKGYLGCQALSEMIQFYLEEVMPQAENQDPDIKAHVNSLGENLKTLRLRLRRCHRFLPCENKSKAVEQVKNAFNKLQEKGIYKAMSEFDIFINYIEAYMTMKIRN

SEQ ID NO: 12 - protein, 150 aa, Homo sapiens
EEVSEYCSHMIGSGHLQSLQRLIDSQMETSCQITFEFVDQEQLKDPVCYLKKAFLLVQDIMEDTMRFRDNTPNAIAIVQLQELSLRLKSCFTKDYEEHDKACVRTFYETPLQLLEKVKNVFNETKNLLDKDWNIFSKNCNNSFAECSSQD

SEQ ID NO: 13 - protein, 340 aa, synthetic construct
SPGQGTQSENSCTHFPGNLPNMLRDLRDAFSRVKTFFQMKDQLDNLLLKESLLEDFKGYLGCQALSEMIQFYLEEVMPQAENQDPDIKAHVNSLGENLKTLRLRLRRCHRFLPCENKSKAVEQVKNAFNKLQEKGIYKAMSEFDIFINYIEAYMTMKIRNGGGGGSGGSGGSGGSGGSGGSGGSGGSGGGEEVSEYCSHMIGSGHLQSLQRLIDSQMETSCQITFEFVDQEQLKDPVCYLKKAFLLVQDIMEDTMRFRDNTPNAIAIVQLQELSLRLKSCFTKDYEEHDKACVRTFYETPLQLLEKVKNVFNETKNLLDKDWNIFSKNCNNSFAECSSQD

SEQ ID NO: 14 - protein, 481 aa, synthetic construct
MTQSENSCTHFPGNLPNMLRDLRDAFSRVKTFFQMKDQLDNLLLKESLLEDFKGYLGCQALSEMIQFYLEEVMPQAENQEPDIKAHVNSLGENLKTLRLRLRRCHRFLPCENKSKAVEQVKNAFNKLQEKGIYKAMSEFDIFINYIEAYMTMNNGGLDYLPNMLRDLRDAFSRVKTFFQMKDQLDNLLLKESLLEDFKGYLGCQALSEMIQFYLEEVMPQAENQDPDIKAHVNSLGENLKTLRLRLRRNHRFLPCENKSKAVEQVKNAFNKLQEKGIYKAMSEFDIFINYIEAYMTMKIRNGGGGGSGGSGGSGGSGGSGGSGGSGGSGGGEEVSEYCSHMIGSGHLQSLQRLIDSQMETSCQITFEFVDQEQLKDPVCYLKKAFLLVQDIMEDTMRFRDNTPNAIAIVQLQELSLRLKSCFTKDYEEHDKACVRTFYETPLQLLEKVKNVFNETKNLLDKDWNIFSKNCNNSFAECSSQD

SEQ ID NO: 15 - protein, 340 aa, synthetic construct
EEVSEYCSHMIGSGHLQSLQRLIDSQMETSCQITFEFVDQEQLKDPVCYLKKAFLLVQDIMEDTMRFRDNTPNAIAIVQLQELSLRLKSCFTKDYEEHDKACVRTFYETPLQLLEKVKNVFNETKNLLDKDWNIFSKNCNNSFAECSSQDGGGGGSGGSGGSGGSGGSGGSGGSGGSGGGSPGQGTQSENSCTHFPGNLPNMLRDLRDAFSRVKTFFQMKDQLDNLLLKESLLEDFKGYLGCQALSEMIQFYLEEVMPQAENQDPDIKAHVNSLGENLKTLRLRLRRCHRFLPCENKSKAVEQVKNAFNKLQEKGIYKAMSEFDIFINYIEAYMTMKIRN

SEQ ID NO: 16 - protein, 481 aa, synthetic construct
EEVSEYCSHMIGSGHLQSLQRLIDSQMETSCQITFEFVDQEQLKDPVCYLKKAFLLVQDIMEDTMRFRDNTPNAIAIVQLQELSLRLKSCFTKDYEEHDKACVRTFYETPLQLLEKVKNVFNETKNLLDKDWNIFSKNCNNSFAECSSQDGGGGGSGGSGGSGGSGGSGGSGGSGGSGGGMTQSENSCTHFPGNLPNMLRDLRDAFSRVKTFFQMKDQLDNLLLKESLLEDFKGYLGCQALSEMIQFYLEEVMPQAENQEPDIKAHVNSLGENLKTLRLRLRRCHRFLPCENKSKAVEQVKNAFNKLQEKGIYKAMSEFDIFINYIEAYMTMNNGGLDYLPNMLRDLRDAFSRVKTFFQMKDQLDNLLLKESLLEDFKGYLGCQALSEMIQFYLEEVMPQAENQDPDIKAHVNSLGENLKTLRLRLRRNHRFLPCENKSKAVEQVKNAFNKLQEKGIYKAMSEFDIFINYIEAYMTMKIRN

SEQ ID NO: 17 - protein, 470 aa, synthetic construct
NKSKAVEQVKNAFNKLQEKGIYKAMSEFDIFINYIEAYMTMNNGGLDYLPNMLRDLRDAFSRVKTFFQMKDQLDNLLLKESLLEDFKGYLGCQALSEMIQFYLEEVMPQAENQDPDIKAHVNSLGENLKTLRLRLRRNHRFLPCENKSKAVEQVKNAFNKLQEKGIYKAMSEFDIFINYIEAYMTMNNGGLDYLPNMLRDLRDAFSRVKTFFQMKDQLDNLLLKESLLEDFKGYLGCQALSEMIQFYLEEVMPQAENQDPDIKAHVNSLGENLKTLRLRLRRNHRFLPCEGGGGGSGGSGGSGGSGGSGGSGGSGGSGGGEEVSEYCSHMIGSGHLQSLQRLIDSQMETSCQITFEFVDQEQLKDPVCYLKKAFLLVQDIMEDTMRFRDNTPNAIAIVQLQELSLRLKSCFTKDYEEHDKACVRTFYETPLQLLEKVKNVFNETKNLLDKDWNIFSKNCNNSFAECSSQD

SEQ ID NO: 18 - protein, 513 aa, synthetic construct
MTAPGAAGRCPPTTWLGSLLLLVCLLASRSITEEVSEYCSHMIGSGHLQSLQRLIDSQMETSCQITFEFVDQEQLKDPVCYLKKAFLLVQDIMEDTMRFRDNTPNAIAIVQLQELSLRLKSCFTKDYEEHDKACVRTFYETPLQLLEKVKNVFNETKNLLDKDWNIFSKNCNNSFAECSSQDGGGGGSGGSGGSGGSGGSGGSGGSGGSGGGMTQSENSCTHFPGNLPNMLRDLRDAFSRVKTFFQMKDQLDNLLLKESLLEDFKGYLGCQALSEMIQFYLEEVMPQAENQEPDIKAHVNSLGENLKTLRLRLRRCHRFLPCENKSKAVEQVKNAFNKLQEKGIYKAMSEFDIFINYIEAYMTMNNGGLDYLPNMLRDLRDAFSRVKTFFQMKDQLDNLLLKESLLEDFKGYLGCQALSEMIQFYLEEVMPQAENQDPDIKAHVNSLGENLKTLRLRLRRNHRFLPCENKSKAVEQVKNAFNKLQEKGIYKAMSEFDIFINYIEAYMTMKIRN

SEQ ID NO: 19 - protein, 481 aa, synthetic construct; identical to SEQ ID NO: 16

SEQ ID NO: 20 - protein, 314 aa, synthetic construct
MTQSENSCTHFPGNLPNMLRDLRDAFSRVKTFFQMKDQLDNLLLKESLLEDFKGYLGCQALSEMIQFYLEEVMPQAENQEPDIKAHVNSLGENLKTLRLRLRRCHRFLPCENKSKAVEQVKNAFNKLQEKGIYKAMSEFDIFINYIEAYMTMNNGGLDYLPNMLRDLRDAFSRVKTFFQMKDQLDNLLLKESLLEDFKGYLGCQALSEMIQFYLEEVMPQAENQDPDIKAHVNSLGENLKTLRLRLRRNHRFLPCENKSKAVEQVKNAFNKLQEKGIYKAMSEFDIFINYIEAYMTMKIRNGGVSGWRLFKKIS

SEQ ID NO: 21 - protein, 486 aa, synthetic construct
EEVSEYCSHMIGSGHLQSLQRLIDSQMETSCQITFEFVDQEQLKDPVCYLKKAFLLVQDIMEDTMRFRDNTPNAIAIVQLQELSLRLKSCFTKDYEEHDKACVRTFYETPLQLLEKVKNVFNETKNLLDKDWNIFSKNCNNSFAECSSQDGGGGGSGGGGSGGSGGSGGSGGSGGSGGSGGSGGGMTQSENSCTHFPGNLPNMLRDLRDAFSRVKTFFQMKDQLDNLLLKESLLEDFKGYLGCQALSEMIQFYLEEVMPQAENQEPDIKAHVNSLGENLKTLRLRLRRCHRFLPCENKSKAVEQVKNAFNKLQEKGIYKAMSEFDIFINYIEAYMTMNNGGLDYLPNMLRDLRDAFSRVKTFFQMKDQLDNLLLKESLLEDFKGYLGCQALSEMIQFYLEEVMPQAENQDPDIKAHVNSLGENLKTLRLRLRRNHRFLPCENKSKAVEQVKNAFNKLQEKGIYKAMSEFDIFINYIEAYMTMKIRN

SEQ ID NO: 22 - protein, 466 aa, synthetic construct
EEVSEYCSHMIGSGHLQSLQRLIDSQMETSCQITFEFVDQEQLKDPVCYLKKAFLLVQDIMEDTMRFRDNTPNAIAIVQLQELSLRLKSCFTKDYEEHDKACVRTFYETPLQLLEKVKNVFNETKNLLDKDWNIFSKNCNNSFAECSSQDGGSGGSGGSGGSGGGMTQSENSCTHFPGNLPNMLRDLRDAFSRVKTFFQMKDQLDNLLLKESLLEDFKGYLGCQALSEMIQFYLEEVMPQAENQEPDIKAHVNSLGENLKTLRLRLRRCHRFLPCENKSKAVEQVKNAFNKLQEKGIYKAMSEFDIFINYIEAYMTMNNGGLDYLPNMLRDLRDAFSRVKTFFQMKDQLDNLLLKESLLEDFKGYLGCQALSEMIQFYLEEVMPQAENQDPDIKAHVNSLGENLKTLRLRLRRNHRFLPCENKSKAVEQVKNAFNKLQEKGIYKAMSEFDIFINYIEAYMTMKIRN

SEQ ID NO: 23 - protein, 327 aa, synthetic construct
EEVSEYCSHMIGSGHLQSLQRLIDSQMETSCQITFEFVDQEQLKDPVCYLKKAFLLVQDIMEDTMRFRDNTPNAIAIVQLQELSLRLKSCFTKDYEEHDKACVRTFYETPLQLLEKVKNVFNETKNLLDKDWNIFSKNCNNSFAECSSQDGGSGGSGGSGGSGGGRASPGQGTQSENSCTHFPGNLPNMLRDLRDAFSRVKTFFQMKDQLDNLLLKESLLEDFKGYLGCQALSEMIQFYLEEVMPQAENQDPDIKAHVNSLGENLKTLRLRLRRCHRFLPCENKSKAVEQVKNAFNKLQEKGIYKAMSEFDIFINYIEAYMTMKIRN

SEQ ID NO: 24 - protein, 337 aa, synthetic construct
EEVSEYCSHMIGSGHLQSLQRLIDSQMETSCQITFEFVDQEQLKDPVCYLKKAFLLVQDIMEDTMRFRDNTPNAIAIVQLQELSLRLKSCFTKDYEEHDKACVRTFYETPLQLLEKVKNVFNETKNLLDKDWNIFSKNCNNSFAECSSQDGGGSGGSGGSGGSGGSGGSGGSGGGRASPGQGTQSENSCTHFPGNLPNMLRDLRDAFSRVKTFFQMKDQLDNLLLKESLLEDFKGYLGCQALSEMIQFYLEEVMPQAENQDPDIKAHVNSLGENLKTLRLRLRRCHRFLPCENKSKAVEQVKNAFNKLQEKGIYKAMSEFDIFINYIEAYMTMKIRN

SEQ ID NO: 25 - protein, 342 aa, synthetic construct
EEVSEYCSHMIGSGHLQSLQRLIDSQMETSCQITFEFVDQEQLKDPVCYLKKAFLLVQDIMEDTMRFRDNTPNAIAIVQLQELSLRLKSCFTKDYEEHDKACVRTFYETPLQLLEKVKNVFNETKNLLDKDWNIFSKNCNNSFAECSSQDGGGGGSGGSGGSGGSGGSGGSGGSGGSGGGRASPGQGTQSENSCTHFPGNLPNMLRDLRDAFSRVKTFFQMKDQLDNLLLKESLLEDFKGYLGCQALSEMIQFYLEEVMPQAENQDPDIKAHVNSLGENLKTLRLRLRRCHRFLPCENKSKAVEQVKNAFNKLQEKGIYKAMSEFDIFINYIEAYMTMKIRN

SEQ ID NO: 26 - protein, 347 aa, synthetic construct
EEVSEYCSHMIGSGHLQSLQRLIDSQMETSCQITFEFVDQEQLKDPVCYLKKAFLLVQDIMEDTMRFRDNTPNAIAIVQLQELSLRLKSCFTKDYEEHDKACVRTFYETPLQLLEKVKNVFNETKNLLDKDWNIFSKNCNNSFAECSSQDGGGGGSGGGGSGGSGGSGGSGGSGGSGGSGGSGGGRASPGQGTQSENSCTHFPGNLPNMLRDLRDAFSRVKTFFQMKDQLDNLLLKESLLEDFKGYLGCQALSEMIQFYLEEVMPQAENQDPDIKAHVNSLGENLKTLRLRLRRCHRFLPCENKSKAVEQVKNAFNKLQEKGIYKAMSEFDIFINYIEAYMTMKIRN

SEQ ID NO: 27 - protein, 5 aa, synthetic construct
GGSGG

SEQ ID NO: 28 - protein, 153 aa, synthetic construct
MTQSENSCTHFPGNLPNMLRDLRDAFSRVKTFFQMKDQLDNLLLKESLLEDFKGYLGCQALSEMIQFYLEEVMPQAENQEPDIKAHVNSLGENLKTLRLRLRRCHRFLPCENKSKAVEQVKNAFNKLQEKGIYKAMSEFDIFINYIEAYMTMN

SEQ ID NO: 29 - protein, 142 aa, synthetic construct
LPNMLRDLRDAFSRVKTFFQMKDQLDNLLLKESLLEDFKGYLGCQALSEMIQFYLEEVMPQAENQDPDIKAHVNSLGENLKTLRLRLRRCHRFLPCENKSKAVEQVKNAFNKLQEKGIYKAMSEFDIFINYIEAYMTMKIRN

SEQ ID NO: 30 - protein, 6 aa, synthetic construct
NGGLDY

SEQ ID NO: 31 - protein, 5 aa, unidentified
YKTIT

SEQ ID NO: 32 - protein, 8 aa, synthetic construct
DKDIRDGD

SEQ ID NO: 33 - protein, 14 aa, synthetic construct
GGSGGSGGSGSGGG

SEQ ID NO: 34 - protein, 24 aa, synthetic construct
GGSGGSGGSGGSGGSGGSGGSGGG

SEQ ID NO: 35 - protein, 30 aa, synthetic construct
GGGGGSGGSGGSGGSGGSGGSGGSGGSGGG

SEQ ID NO: 36 - protein, 35 aa, synthetic construct
GGGGGSGGGGSGGSGGSGGSGGSGGSGGSGGSGGG

SEQ ID NO: 37 - protein, 141 aa, synthetic construct
CTHFPGNLPNMLRDLRDAFSRVKTFFQMKDQLDNLLLKESLLEDFKGYLGCQALSEMIQFYLEEVMPQAENQDPDIKAHVNSLGENLKTLRLRLRRCHRFLPCENKSKAVEQVKNAFNKLQEKGIYKAMSEFDIFINYIEA

SEQ ID NO: 38 - protein, 136 aa, synthetic construct
NMLRDLRDAFSRVKTFFQMKDQLDNLLLKESLLEDFKGYLGCQALSEMIQFYLEEVMPQAENQDPDIKAHVNSLGENLKTLRLRLRRCHRFLPCENKSKAVEQVKNAFNKLQEKGIYKAMSEFDIFINYIEAYMTM

SEQ ID NO: 39 - protein, 152 aa, synthetic construct
MTQSENSCTHFOGNLPNMLRDLRDAFSRVKTFFQMKDQLDNLLLKESLLEDFKGYLGCQALSEMIQFYLEEVMPQAENQDPDIKAHVNSLGENLKTLRLRLRRCHRFLPCENKSKAVEQVKNAFNKLQEKGIYKAMSEFDIFINYIEAMTMN

SEQ ID NO: 40 - protein, 138 aa, synthetic construct
LPNMLRDLRDAFSRVKTFFQMKDQLDNLLLKESLLEDFKGYLGCQALSEMIQFYLEEVMPQAENQDPDIKAHVNSLGENLKTLRLRLRRCHRFLPCENKSKAVEQVKNAFNKLQEKGIYKAMSEFDIFINYIEAYMTM

SEQ ID NO: 41 - protein, 150 aa, synthetic construct
MTQSENSCTHFOGNLPNMLRDLRDAFSRVKTFFQMKDQLDNLLLKESLLEDFKGYLGCQALSEMIQFYLEEVMPQAENQDPDIKAHVNSLGENLKTLRLRLRRCHRFLPCENKSKAVEQVKNAFNKLQEKGIYKAMSEFDIFINYIEAYL

SEQ ID NO: 42 - protein, 140 aa, synthetic construct
PEFANMLRDLRDAFSRVKTFFQMKDQLDNLLLKESLLEDFKGYLGCQALSEMIQFYLEEVMPQAENQDPDIKAHVNSLGENLKTLRLRLRRCHRFLPCENKSKAVEQVKNAFNKLQEKGIYKAMSEFDIFINYIEAYMTM

SEQ ID NO: 43 - protein, 149 aa, synthetic construct
MTQSENSCTHFPGNLPNMLRDLRDAFSRVKTFFQMKDQLDNLLLKESLLEDFKGYLGCQALSEMIQFYLEEVMPQAENQDPDIKAHVNSLGENLKTLRLRLRRCHRFLPCENKSKAVEQVKNAFNKLQEKGIYKAMSEFDIFINYIEAK

SEQ ID NO: 44 - protein, 139 aa, synthetic construct
ELANMLRDLRDAFSRVKTFFQMKDQLDNLLLKESLLEDFKGYLGCQALSEMIQFYLEEVMPQAENQDPDIKAHVNSLGENLKTLRLRLRRCHRFLPCENKSKAVEQVKNAFNKLQEKGIYKAMSEFDIFINYIEAYMTM

SEQ ID NO: 45 - protein, 8 aa, synthetic construct
NFGGLDYL

SEQ ID NO: 46 - protein, 10 aa, synthetic construct
LYKTITPEFA

SEQ ID NO: 47 - protein, 12 aa, synthetic construct
KDKDIRDGDELA

SEQ ID NO: 48 - protein, 6 aa, synthetic construct
FGGLDY

SEQ ID NO: 49 - protein, 308 aa, synthetic construct
MTQSENSCTHFPGNLPNMLRDLRDAFSRVKTFFQMKDQLDNLLLKESLLEDFKGYLGCQALSEMIQFYLEEVMPQAENQDPDIKAHVNSLGENLKTLRLRLRRCHRFLPCENKSKAVEQVKNAFNKLQEKGIYKAMSEFDIFINYIEAYLYKTITPEFANMLRDLRDAFSRVKTFFQMKDQLDNLLLKESLLEDFKGYLGCQALSEMIQFYLEEVMPQAENQDPDIKAHVNSLGENLKTLRLRLRRCHRFLPCENKSKAVEQVKNAFNKLQEKGIYKAMSEFDIFINYIEAYMTMGGVSGWRLFKKIS

SEQ ID NO: 50 - protein, 173 aa, synthetic construct
SPGQGTQSENSCTHFPGNLPNMLRDLRDAFSRVKTFFQMKDQLDNLLLKESLLEDFKGYLGCQALSEMIQFYLEEVMPQAENQDPDIKAHVNSLGENLKTLRLRLRRCHRFLPCENKSKAVEQVKNAFNKLQEKGIYKAMSEFDIFINYIEAYMTMKIRNGGVSGWRLFKKIS

SEQ ID NO: 51 - protein, 163 aa, synthetic construct
EEVSEYCSHMIGSGHLQSLQRLIDSQMETSCQITFEFVDQEQLKDPVCYLKKAFLLVQDIMEDTMRFRDNTPNAIAIVQLQELSLRLKSCFTKDYEEHDKACVRTFYETPLQLLEKVKNVFNETKNLLDKDWNIFSKNCNNSFAECSSQDGGVSGWRLFKKIS

SEQ ID NO: 52 - protein, 353 aa, synthetic construct
SPGQGTQSENSCTHFPGNLPNMLRDLRDAFSRVKTFFQMKDQLDNLLLKESLLEDFKGYLGCQALSEMIQFYLEEVMPQAENQDPDIKAHVNSLGENLKTLRLRLRRCHRFLPCENKSKAVEQVKNAFNKLQEKGIYKAMSEFDIFINYIEAYMTMKIRNGGGGGSGGSGGSGGSGGSGGSGGSGGSGGGEEVSEYCSHMIGSGHLQSLQRLIDSQMETSCQITFEFVDQEQLKDPVCYLKKAFLLVQDIMEDTMRFRDNTPNAIAIVQLQELSLRLKSCFTKDYEEHDKACVRTFYETPLQLLEKVKNVFNETKNLLDKDWNIFSKNCNNSFAECSSQDGGVSGWRLFKKIS

SEQ ID NO: 53 - protein, 494 aa, synthetic construct
MTQSENSCTHFPGNLPNMLRDLRDAFSRVKTFFQMKDQLDNLLLKESLLEDFKGYLGCQALSEMIQFYLEEVMPQAENQEPDIKAHVNSLGENLKTLRLRLRRCHRFLPCENKSKAVEQVKNAFNKLQEKGIYKAMSEFDIFINYIEAYMTMNNGGLDYLPNMLRDLRDAFSRVKTFFQMKDQLDNLLLKESLLEDFKGYLGCQALSEMIQFYLEEVMPQAENQDPDIKAHVNSLGENLKTLRLRLRRNHRFLPCENKSKAVEQVKNAFNKLQEKGIYKAMSEFDIFINYIEAYMTMKIRNGGGGGSGGSGGSGGSGGSGGSGGSGGSGGGEEVSEYCSHMIGSGHLQSLQRLIDSQMETSCQITFEFVDQEQLKDPVCYLKKAFLLVQDIMEDTMRFRDNTPNAIAIVQLQELSLRLKSCFTKDYEEHDKACVRTFYETPLQLLEKVKNVFNETKNLLDKDWNIFSKNCNNSFAECSSQDGGVSGWRLFKKIS

SEQ ID NO: 54 - protein, 353 aa, synthetic construct
EEVSEYCSHMIGSGHLQSLQRLIDSQMETSCQITFEFVDQEQLKDPVCYLKKAFLLVQDIMEDTMRFRDNTPNAIAIVQLQELSLRLKSCFTKDYEEHDKACVRTFYETPLQLLEKVKNVFNETKNLLDKDWNIFSKNCNNSFAECSSQDGGGGGSGGSGGSGGSGGSGGSGGSGGSGGGSPGQGTQSENSCTHFPGNLPNMLRDLRDAFSRVKTFFQMKDQLDNLLLKESLLEDFKGYLGCQALSEMIQFYLEEVMPQAENQDPDIKAHVNSLGENLKTLRLRLRRCHRFLPCENKSKAVEQVKNAFNKLQEKGIYKAMSEFDIFINYIEAYMTMKIRNGGVSGWRLFKKIS

SEQ ID NO: 55 - skipped

SEQ ID NO: 56 - protein, 484 aa, synthetic construct
NKSKAVEQVKNAFNKLQEKGIYKAMSEFDIFINYIEAYMTMNNGGLDYLPNMLRDLRDAFSRVKTFFQMKDQLDNLLLKESLLEDFKGYLGCQALSEMIQFYLEEVMPQAENQDPDIKAHVNSLGENLKTLRLRLRRNHRFLPCENKSKAVEQVKNAFNKLQEKGIYKAMSEFDIFINYIEAYMTMNNGGLDYLPNMLRDLRDAFSRVKTFFQMKDQLDNLLLKESLLEDFKGYLGCQALSEMIQFYLEEVMPQAENQDPDIKAHVNSLGENLKTLRLRLRRNHRFLPCEGGGGGSGGSGGSGGSGGSGGSGGSGGSGGGEEVSEYCSHMIGSGHLQSLQRLIDSQMETSCQITFEFVDQEQLKDPVCYLKKAFLLVQDIMEDTMRFRDNTPNAIAIVQLQELSLRLKSCFTKDYEEHDKACVRTFYETPLQLLEKVKNVFNETKNLLDKDWNIFSKNCNNSFAECSSQDGGGVSGWRLFKKIS

SEQ ID NO: 57 - protein, 526 aa, synthetic construct
MTAPGAAGRCPPTTWLGSLLLLVCLLASRSITEEVSEYCSHMIGSGHLQSLQRLIDSQMETSCQITFEFVDQEQLKDPVCYLKKAFLLVQDIMEDTMRFRDNTPNAIAIVQLQELSLRLKSCFTKDYEEHDKACVRTFYETPLQLLEKVKNVFNETKNLLDKDWNIFSKNCNNSFAECSSQDGGGGGSGGSGGSGGSGGSGGSGGSGGSGGGMTQSENSCTHFPGNLPNMLRDLRDAFSRVKTFFQMKDQLDNLLLKESLLEDFKGYLGCQALSEMIQFYLEEVMPQAENQEPDIKAHVNSLGENLKTLRLRLRRCHRFLPCENKSKAVEQVKNAFNKLQEKGIYKAMSEFDIFINYIEAYMTMNNGGLDYLPNMLRDLRDAFSRVKTFFQMKDQLDNLLLKESLLEDFKGYLGCQALSEMIQFYLEEVMPQAENQDPDIKAHVNSLGENLKTLRLRLRRNHRFLPCENKSKAVEQVKNAFNKLQEKGIYKAMSEFDIFINYIEAYMTMKIRNGGVSGWRLFKKIS

SEQ ID NO: 58 - protein, 494 aa, synthetic construct
EEVSEYCSHMIGSGHLQSLQRLIDSQMETSCQITFEFVDQEQLKDPVCYLKKAFLLVQDIMEDTMRFRDNTPNAIAIVQLQELSLRLKSCFTKDYEEHDKACVRTFYETPLQLLEKVKNVFNETKNLLDKDWNIFSKNCNNSFAECSSQDGGGGGSGGSGGSGGSGGSGGSGGSGGSGGGMTQSENSCTHFPGNLPNMLRDLRDAFSRVKTFFQMKDQLDNLLLKESLLEDFKGYLGCQALSEMIQFYLEEVMPQAENQEPDIKAHVNSLGENLKTLRLRLRRCHRFLPCENKSKAVEQVKNAFNKLQEKGIYKAMSEFDIFINYIEAYMTMNNGGLDYLPNMLRDLRDAFSRVKTFFQMKDQLDNLLLKESLLEDFKGYLGCQALSEMIQFYLEEVMPQAENQDPDIKAHVNSLGENLKTLRLRLRRNHRFLPCENKSKAVEQVKNAFNKLQEKGIYKAMSEFDIFINYIEAYMTMKIRNGGVSGWRLFKKIS

SEQ ID NO: 59 - protein, 499 aa, synthetic construct
EEVSEYCSHMIGSGHLQSLQRLIDSQMETSCQITFEFVDQEQLKDPVCYLKKAFLLVQDIMEDTMRFRDNTPNAIAIVQLQELSLRLKSCFTKDYEEHDKACVRTFYETPLQLLEKVKNVFNETKNLLDKDWNIFSKNCNNSFAECSSQDGGGGGSGGGGSGGSGGSGGSGGSGGSGGSGGSGGGMTQSENSCTHFPGNLPNMLRDLRDAFSRVKTFFQMKDQLDNLLLKESLLEDFKGYLGCQALSEMIQFYLEEVMPQAENQEPDIKAHVNSLGENLKTLRLRLRRCHRFLPCENKSKAVEQVKNAFNKLQEKGIYKAMSEFDIFINYIEAYMTMNNGGLDYLPNMLRDLRDAFSRVKTFFQMKDQLDNLLLKESLLEDFKGYLGCQALSEMIQFYLEEVMPQAENQDPDIKAHVNSLGENLKTLRLRLRRNHRFLPCENKSKAVEQVKNAFNKLQEKGIYKAMSEFDIFINYIEAYMTMKIRNGGVSGWRLFKKIS

SEQ ID NO: 60 - protein, 479 aa, synthetic construct
EEVSEYCSHMIGSGHLQSLQRLIDSQMETSCQITFEFVDQEQLKDPVCYLKKAFLLVQDIMEDTMRFRDNTPNAIAIVQLQELSLRLKSCFTKDYEEHDKACVRTFYETPLQLLEKVKNVFNETKNLLDKDWNIFSKNCNNSFAECSSQDGGSGGSGGSGGSGGGMTQSENSCTHFPGNLPNMLRDLRDAFSRVKTFFQMKDQLDNLLLKESLLEDFKGYLGCQALSEMIQFYLEEVMPQAENQEPDIKAHVNSLGENLKTLRLRLRRCHRFLPCENKSKAVEQVKNAFNKLQEKGIYKAMSEFDIFINYIEAYMTMNNGGLDYLPNMLRDLRDAFSRVKTFFQMKDQLDNLLLKESLLEDFKGYLGCQALSEMIQFYLEEVMPQAENQDPDIKAHVNSLGENLKTLRLRLRRNHRFLPCENKSKAVEQVKNAFNKLQEKGIYKAMSEFDIFINYIEAYMTMKIRNGGVSGWRLFKKIS

SEQ ID NO: 61 - protein, 340 aa, unidentified
EEVSEYCSHMIGSGHLQSLQRLIDSQMETSCQITFEFVDQEQLKDPVCYLKKAFLLVQDIMEDTMRFRDNTPNAIAIVQLQELSLRLKSCFTKDYEEHDKACVRTFYETPLQLLEKVKNVFNETKNLLDKDWNIFSKNCNNSFAECSSQDGGSGGSGGSGGSGGGRASPGQGTQSENSCTHFPGNLPNMLRDLRDAFSRVKTFFQMKDQLDNLLLKESLLEDFKGYLGCQALSEMIQFYLEEVMPQAENQDPDIKAHVNSLGENLKTLRLRLRRCHRFLPCENKSKAVEQVKNAFNKLQEKGIYKAMSEFDIFINYIEAYMTMKIRNGGVSGWRLFKKIS

SEQ ID NO: 62 - protein, 350 aa, synthetic construct
EEVSEYCSHMIGSGHLQSLQRLIDSQMETSCQITFEFVDQEQLKDPVCYLKKAFLLVQDIMEDTMRFRDNTPNAIAIVQLQELSLRLKSCFTKDYEEHDKACVRTFYETPLQLLEKVKNVFNETKNLLDKDWNIFSKNCNNSFAECSSQDGGGSGGSGGSGGSGGSGGSGGSGGGRASPGQGTQSENSCTHFPGNLPNMLRDLRDAFSRVKTFFQMKDQLDNLLLKESLLEDFKGYLGCQALSEMIQFYLEEVMPQAENQDPDIKAHVNSLGENLKTLRLRLRRCHRFLPCENKSKAVEQVKNAFNKLQEKGIYKAMSEFDIFINYIEAYMTMKIRNGGVSGWRLFKKIS

SEQ ID NO: 63 - protein, 355 aa, synthetic construct
EEVSEYCSHMIGSGHLQSLQRLIDSQMETSCQITFEFVDQEQLKDPVCYLKKAFLLVQDIMEDTMRFRDNTPNAIAIVQLQELSLRLKSCFTKDYEEHDKACVRTFYETPLQLLEKVKNVFNETKNLLDKDWNIFSKNCNNSFAECSSQDGGGGGSGGSGGSGGSGGSGGSGGSGGSGGGRASPGQGTQSENSCTHFPGNLPNMLRDLRDAFSRVKTFFQMKDQLDNLLLKESLLEDFKGYLGCQALSEMIQFYLEEVMPQAENQDPDIKAHVNSLGENLKTLRLRLRRCHRFLPCENKSKAVEQVKNAFNKLQEKGIYKAMSEFDIFINYIEAYMTMKIRNGGVSGWRLFKKIS

SEQ ID NO: 64 - protein, 360 aa, synthetic construct
EEVSEYCSHMIGSGHLQSLQRLIDSQMETSCQITFEFVDQEQLKDPVCYLKKAFLLVQDIMEDTMRFRDNTPNAIAIVQLQELSLRLKSCFTKDYEEHDKACVRTFYETPLQLLEKVKNVFNETKNLLDKDWNIFSKNCNNSFAECSSQDGGGGGSGGGGSGGSGGSGGSGGSGGSGGSGGSGGGRASPGQGTQSENSCTHFPGNLPNMLRDLRDAFSRVKTFFQMKDQLDNLLLKESLLEDFKGYLGCQALSEMIQFYLEEVMPQAENQDPDIKAHVNSLGENLKTLRLRLRRCHRFLPCENKSKAVEQVKNAFNKLQEKGIYKAMSEFDIFINYIEAYMTMKIRNGGVSGWRLFKKIS

SEQ ID NO: 65 - protein, 149 aa, synthetic construct
MTQSENSCTHFPGNLPNMLRDLRDAFSRVKTFFQMKDQLDNLLLKESLLEDFKGYLGCQALSEMIQFYLEEVMPQAENQDPDIKAHVNSLGENLKTLRLRLRRCHRFLPCENKSKAVEQVKNAFNKLQEKGIYKAMSEFDIFINYIEAY

SEQ ID NO: 66 - protein, 140 aa, synthetic construct
NMLRDLRDAFSRVKTFFQMKDQLDNLLLKESLLEDFKGYLGCQALSEMIQFYLEEVMPQAENQDPDIKAHVNSLGENLKTLRLRLRRCHRFLPCENKSKAVEQVKNAFNKLQEKGIYKAMSEFDIFINYIEAYMTMKIRN

SEQ ID NO: 67 - protein, 4 aa, synthetic construct
MTMN

SEQ ID NO: 68 - protein, 4 aa, synthetic construct
PEFA

SEQ ID NO: 69 - protein, 18 aa, synthetic construct
MHSSALLCCLVLLTGVRA

SEQ ID NO: 70 - protein, 32 aa, synthetic construct
MTAPGAAGRCPPTTWLGSLLLLVCLLASRSIT

SEQ ID NO: 71 - protein, 8 aa, synthetic construct
NNGGLDYL

SEQ ID NO: 72 - protein, 511 aa, synthetic construct
  source 1..511: note = CSF1-Foldikine10-TEV-his-hibit
EEVSEYCSHMIGSGHLQSLQRLIDSQMETSCQITFEFVDQEQLKDPVCYLKKAFLLVQDIMEDTMRFRDNTPNAIAIVQLQELSLRLKSCFTKDYEEHDKACVRTFYETPLQLLEKVKNVFNETKNLLDKDWNIFSKNCNNSFAECSSQDGGGGGSGGSGGSGGSGGSGGSGGSGGSGGGMTQSENSCTHFPGNLPNMLRDLRDAFSRVKTFFQMKDQLDNLLLKESLLEDFKGYLGCQALSEMIQFYLEEVMPQAENQEPDIKAHVNSLGENLKTLRLRLRRCHRFLPCENKSKAVEQVKNAFNKLQEKGIYKAMSEFDIFINYIEAYMTMNNGGLDYLPNMLRDLRDAFSRVKTFFQMKDQLDNLLLKESLLEDFKGYLGCQALSEMIQFYLEEVMPQAENQDPDIKAHVNSLGENLKTLRLRLRRNHRFLPCENKSKAVEQVKNAFNKLQEKGIYKAMSEFDIFINYIEAYMTMKIRNGENLYFQSGGHHHHHHGGGVSGWRLFKKIS

SEQ ID NO: 73 - protein, 511 aa, synthetic construct
  source 1..511: note = CSF1(E82A)-Foldikine10-TEV-his-hibit
EEVSEYCSHMIGSGHLQSLQRLIDSQMETSCQITFEFVDQEQLKDPVCYLKKAFLLVQDIMEDTMRFRDNTPNAIAIVQLQALSLRLKSCFTKDYEEHDKACVRTFYETPLQLLEKVKNVFNETKNLLDKDWNIFSKNCNNSFAECSSQDGGGGGSGGSGGSGGSGGSGGSGGSGGSGGGMTQSENSCTHFPGNLPNMLRDLRDAFSRVKTFFQMKDQLDNLLLKESLLEDFKGYLGCQALSEMIQFYLEEVMPQAENQEPDIKAHVNSLGENLKTLRLRLRRCHRFLPCENKSKAVEQVKNAFNKLQEKGIYKAMSEFDIFINYIEAYMTMNNGGLDYLPNMLRDLRDAFSRVKTFFQMKDQLDNLLLKESLLEDFKGYLGCQALSEMIQFYLEEVMPQAENQDPDIKAHVNSLGENLKTLRLRLRRNHRFLPCENKSKAVEQVKNAFNKLQEKGIYKAMSEFDIFINYIEAYMTMKIRNGENLYFQSGGHHHHHHGGGVSGWRLFKKIS

SEQ ID NO: 74 - protein, 370 aa, synthetic construct
EEVSEYCSHMIGSGHLQSLQRLIDSQMETSCQITFEFVDQEQLKDPVCYLKKAFLLVQDIMEDTMRFRDNTPNAIAIVQLQELSLRLKSCFTKDYEEHDKACVRTFYETPLQLLEKVKNVFNETKNLLDKDWNIFSKNCNNSFAECSSQDGGGGGSGGSGGSGGSGGSGGSGGSGGSGGGSPGQGTQSENSCTHFPGNLPNMLRDLRDAFSRVKTFFQMKDQLDNLLLKESLLEDFKGYLGCQALSEMIQFYLEEVMPQAENQDPDIKAHVNSLGENLKTLRLRLRRCHRFLPCENKSKAVEQVKNAFNKLQEKGIYKAMSEFDIFINYIEAYMTMKIRNGENLYFQSGGHHHHHHGGGVSGWRLFKKIS